European Patent Specification EP 3 797 582 B1, published December 17, 2025. Title: LETTUCE PLANTS HAVING RESISTANCE TO NASONOVIA RIBISNIGRI BIOTYPE NR:1. Applicant: Seminis Vegetable Seeds, Inc. The sequence listing filed with the application follows.

SEQUENCE LISTING (95 sequences)

SEQ ID NO: 1 - DNA, 121 bp, Lactuca serriola
acaagttgaaatcactatatggttgtggtattaattcccttgataatctagcaaatgaagtcaatggaaattcacagtcaacactcgaacatcttaattctcaagtctcccaaaattcttc

SEQ ID NO: 2 - DNA, 31 bp, Artificial Sequence
  Primer
cactatatggttgtggtattaattcccttga

SEQ ID NO: 3 - DNA, 27 bp, Artificial Sequence
  Primer
gggagacttgagaattaagatgttcga

SEQ ID NO: 4 - DNA, 20 bp, Artificial Sequence
  Probe
tgaatttccattgacttcat

SEQ ID NO: 5 - DNA, 18 bp, Artificial Sequence
  Probe
aatttccattggcttcat

SEQ ID NO: 6 - DNA, 121 bp, Lactuca serriola
gagatatgaccgattaaggagtatttctggaaggattcagacggttgttggtgatttggcaacacaaggagagaggcttcagtctttgctgagctggcgagatcccagagcaactgcattg

SEQ ID NO: 7 - DNA, 27 bp, Artificial Sequence
  Primer
accgattaaggagtatttctggaagga

SEQ ID NO: 8 - DNA, 22 bp, Artificial Sequence
  Primer
cagcaaagactgaagcctctct

SEQ ID NO: 9 - DNA, 19 bp, Artificial Sequence
  Probe
tggtgatttggcaacacaa

SEQ ID NO: 10 - DNA, 20 bp, Artificial Sequence
  Probe
ttggtgatttggctacacaa

SEQ ID NO: 11 - DNA, 121 bp, Lactuca serriola
  misc_feature (4)..(4): n is a, c, g, or t
  misc_feature (100)..(100): n is a, c, g, or t
cacnccatactctacctctacaccataactactacaatcagacgccgccgtaaacaaccacctatcggcattcaactccgtcgtcgactccgttcgcttngcaaaccggcctttgatcctc

SEQ ID NO: 12 - DNA, 18 bp, Artificial Sequence
  Primer
aatcagacgccgccgtaa

SEQ ID NO: 13 - DNA, 19 bp, Artificial Sequence
  Primer
gagtcgacgacggagttga

SEQ ID NO: 14 - DNA, 18 bp, Artificial Sequence
  Probe
atgccgataggtggttgt

SEQ ID NO: 15 - DNA, 17 bp, Artificial Sequence
  Probe
tgccgatagctggttgt

SEQ ID NO: 16 - DNA, 201 bp, Lactuca serriola
cattgtcagttgtgccctaggccatttcacagtccctttgatgcaagattccttaatggcagacattttgccactctaaacgtccaaatttgtgatttcatatcctcgaaacttcaagtctgttggctcaattctggaggaaatgttggaaaaggttcctcttgacaatacaatattgagggagtatcagaagttaccatc

SEQ ID NO: 17 - DNA, 24 bp, Artificial Sequence
  Primer
gccactctaaacgtccaaatttgt

SEQ ID NO: 18 - DNA, 25 bp, Artificial Sequence
  Primer
cagaattgagccaacagacttgaag

SEQ ID NO: 19 - DNA, 18 bp, Artificial Sequence
  Probe
tttcgaggatatgaaatc

SEQ ID NO: 20 - DNA, 15 bp, Artificial Sequence
  Probe
cgaggatctgaaatc

SEQ ID NO: 21 - DNA, 121 bp, Lactuca serriola
  misc_feature (16)..(16): n is a, c, g, or t
tactccaatagggggngggcgggtcaacccgcccgatagaagaaaccctaatagcccaaatatattcaatgggcccacttctcaccccaaagaacaatctgacttggtcaacgctctttcc

SEQ ID NO: 22 - DNA, 20 bp, Artificial Sequence
  Primer
cccgcccgatagaagaaacc

SEQ ID NO: 23 - DNA, 19 bp, Artificial Sequence
  Primer
ggtgagaagtgggcccatt

SEQ ID NO: 24 - DNA, 18 bp, Artificial Sequence
  Probe
aatagcccaaatatattc

SEQ ID NO: 25 - DNA, 16 bp, Artificial Sequence
  Probe
tagcccaaacatattc

SEQ ID NO: 26 - DNA, 201 bp, Lactuca serriola
gtcctgtcctgtaaagtgtcaaccgacttacccttttaatggttcaacagattcccacactcgaggctccgcatctttgtccttacatatctttaaaaacaaaaaataaaaataaaaattagaactttgaaaagaaaaaaacgtgtatttgttgttaatatcaaattttcatacttggagtccagaaacactatcggttgc

SEQ ID NO: 27 - DNA, 21 bp, Artificial Sequence
  Primer
ggctccgcatctttgtcctta

SEQ ID NO: 28 - DNA, 34 bp, Artificial Sequence
  Primer
caacaaatacacgtttttttcttttcaaagttct

SEQ ID NO: 29 - DNA, 23 bp, Artificial Sequence
  Probe
catatctttaaaaacaaaaaata

SEQ ID NO: 30 - DNA, 20 bp, Artificial Sequence
  Probe
atctttaaaaaccaaaaata

SEQ ID NO: 31 - DNA, 432 bp, Lactuca serriola
  misc_feature (273)..(273): n is a, c, g, or t
  misc_feature (298)..(298): n is a, c, g, or t
  misc_feature (348)..(348): n is a, c, g, or t
cgaaggacacgagcttgggtctggtttgatcggaaaggctcaagggtattatgtatcgagttccatagatgggaagagtcagacgatggcgtttactgtgatgtttatgcacgggagttatattgatagtttgagctttatgggggttcaccggagtgcggtggcggagtcccagctggcggtgatgggtggcaccgggaagtatgtgaatgctaaagggcatgcggtggtgaagacttttcaggggacaaaccagcagaataatgatggaantgagacactgcttcagtttcatgtntatcttgcgtattagtttgtataagtctatgtgtgtttggtttctatttntatgctttccatgtttatgtgatgttatgaaaatttgtgtgtgaaatacaaaagaatttaacaatttctacttttcccggagag

SEQ ID NO: 32 - DNA, 17 bp, Artificial Sequence
  Primer
agtcccagctggcggtg

SEQ ID NO: 33 - DNA, 24 bp, Artificial Sequence
  Primer
ccatcattattctgctggtttgtc

SEQ ID NO: 34 - DNA, 14 bp, Artificial Sequence
  Probe
cttcccggtgccac

SEQ ID NO: 35 - DNA, 14 bp, Artificial Sequence
  Probe
cttcccagtgccac

SEQ ID NO: 36 - DNA, 121 bp, Lactuca serriola
agaggccaatgtgttgaagatcaggaaagtttatgatgcatttttggctgaatttcctctctgttatggctactggaagaagtatgctgatcatgaagcaagattggggtctattgataaa

SEQ ID NO: 37 - DNA, 25 bp, Artificial Sequence
  Primer
aaagtttatgatgcatttttggctg

SEQ ID NO: 38 - DNA, 26 bp, Artificial Sequence
  Primer
ttgcttcatgatcagcatacttcttc

SEQ ID NO: 39 - DNA, 18 bp, Artificial Sequence
  Probe
atttcctctctgttatgg

SEQ ID NO: 40 - DNA, 17 bp, Artificial Sequence
  Probe
tttcctctgtgttatgg

SEQ ID NO: 41 - DNA, 2003 bp, Lactuca serriola
  misc_feature (52)..(52): n is a, c, g, or t
  misc_feature (178)..(178): n is a, c, g, or t
  misc_feature (211)..(211): n is a, c, g, or t
  misc_feature (232)..(232): n is a, c, g, or t
  misc_feature (386)..(386): n is a, c, g, or t
  misc_feature (648)..(648): n is a, c, g, or t
  misc_feature (662)..(662): n is a, c, g, or t
  misc_feature (690)..(690): n is a, c, g, or t
  misc_feature (733)..(733): n is a, c, g, or t
  misc_feature (912)..(912): n is a, c, g, or t
  misc_feature (936)..(936): n is a, c, g, or t
  misc_feature (991)..(991): n is a, c, g, or t
  misc_feature (1015)..(1015): n is a, c, g, or t
  misc_feature (1033)..(1033): n is a, c, g, or t
  misc_feature (1052)..(1052): n is a, c, g, or t
  misc_feature (1062)..(1062): n is a, c, g, or t
  misc_feature (1099)..(1099): n is a, c, g, or t
  misc_feature (1169)..(1169): n is a, c, g, or t
  misc_feature (1182)..(1182): n is a, c, g, or t
  misc_feature (1213)..(1213): n is a, c, g, or t
  misc_feature (1238)..(1238): n is a, c, g, or t
  misc_feature (1244)..(1244): n is a, c, g, or t
  misc_feature (1252)..(1252): n is a, c, g, or t
  misc_feature (1265)..(1265): n is a, c, g, or t
  misc_feature (1283)..(1283): n is a, c, g, or t
  misc_feature (1329)..(1329): n is a, c, g, or t
  misc_feature (1344)..(1344): n is a, c, g, or t
  misc_feature (1690)..(1690): n is a, c, g, or t
  misc_feature (1833)..(1833): n is a, c, g, or t
cgggggctagtgagttacgttccgtcgtacctcgccggaaaacattcactgncgccataaactacggtgttgcagaaatagttgctctaggtgtgaaggaaagttatcactcggtggttattggatctataagcttgcatctttgaatctctgttcgcacttttcactttctctctcnagaaaatgaggacggatatggtgaataggtgtntgagtttatcacaacattcgnttccacaatcaccttcttcttcgtcttctccttcttcttcattgcaaactctagcctctgcaatctcttcaccgtcagcaaaacgacggtgtttgacccaccgcgcactggcttaccgctacgttcaccggtcggcgatatttgggacgaagcngaagagatccgacccatctagagagccgcagcttatccaacgcaccgtctccgccagcttagatgcagagttttcggatgaagaattctcaaagaaaattcgagaactagctctccagtttcaagtttccgacgaatttggcaataaagagaagtatgacggtttagcattggaattggaattggcatcggagagccagagcccatttgctggtttgaagatggaagtgcctgactggccaggggatatgattccggcgagnattgagcgaaaggngaacagcgttgagttgccattttcattncgaattatcaagaggaagaaacaatggcaggagggaataaganacgcaggtgaatctgcctattgttcagtaaaaaaagctttctcttcaatggtgttcataatccgagagcttcaaagctacacacttcaaatgagagagcttttatactacgaagatttacaggggattcttgtgagagttcagcaagaaatgaacgcatctttcgtctggttgttccancaagtcttttcccaaacccctacnttaatggtgtacgtgatgattcttttagccaattacagtgtatattcaatgtcanacaatatcgcactcgcggcgccgncacctcccgccaccgtanagtcgattacagaacaccnaagtgaaacnaaattcgattcttcatcagtcaaaacgttttctgtanattcaggtgggaaaaccacctcaatcggcggaaacaacggcggcggtgggaaattcagggcagttgctancgggacagacggngacgggagatttgatggatctataacttcancgtcatcaatcgtaaacccgacaangactancgaggagncggtttcgggtcnagcgagtaaggataatgnatgggagtcatggaattcgattgtggatgaagctgacagaatgcanggtgtgatcggaganaacggcgatctggatcatgaaactatgaaaagatttgtttctccggtgactgtgaaaatcgaggaagaagatacagaagatcactccaaaacagagcttctttatcaaacgggtctctcacaagaacccgacaacccgcttcttcttgcgaattacgcccagtttctgtacctcgttacacgagattacgatagagctgaggattacttcaaaagagcttcaatggtggaacctaaagacgcagaagcacttaacaaatacgcaagctttttatggcaagttcgaaaagacttgtgggctgctgaagagacttatttggaagccatttctgctgatcctacaaacnctttttatgctgcaaattatgcacatttcttatggagcaccggtggagaagacacttgtttccctcttgactcgccgggaaatatgttctccgacgaagtgtgaattaaccaccggcgtcggagacgtgggtttaacttaganagttgggacatgataataaacgagatttgagcgggaagtggtggtggatggttgaaaggtggaatatgataatcttgattttccggcgaaaggtggtttgaagttgtcaaaaattgtaattaagttttgttgatatcaaattataaatgaaaatgaatttaggtgaaacg

SEQ ID NO: 42 - DNA, 21 bp, Artificial Sequence
  Primer
catctagagagccgcagctta

SEQ ID NO: 43 - DNA, 26 bp, Artificial Sequence
  Primer
attcttcatccgaaaactctgcatct

SEQ ID NO: 44 - DNA, 16 bp, Artificial Sequence
  Probe
tccaacgcaccgtctc

SEQ ID NO: 45 - DNA, 14 bp, Artificial Sequence
  Probe
caacgcgccgtctc

SEQ ID NO: 46 - DNA, 201 bp, Lactuca serriola
tggcttaggagatgggaaagaacgaaggtcaactgctcaccatagaactcttgctaaacaggttgattcgtcaccatcaaattaaacatgagttcacaattctggggtagggatctgattttcctagatgataatgacgagaatgatggtgattcaagagacctatgctttggggaaagggtctatgggattttttatttt

SEQ ID NO: 47 - DNA, 25 bp, Artificial Sequence
  Primer
gctaaacaggttgattcgtcaccat

SEQ ID NO: 48 - DNA, 29 bp, Artificial Sequence
  Primer
accatcattctcgtcattatcatctagga

SEQ ID NO: 49 - DNA, 14 bp, Artificial Sequence
  Probe
accccagaattgtg

SEQ ID NO: 50 - DNA, 14 bp, Artificial Sequence
  Probe
accccaggattgtg

SEQ ID NO: 51 - DNA, 201 bp, Lactuca serriola
aaaagaatttgctaaccctgaagctaaaataaaaggtctttcatgtctccactgttcaaaagttcatttttgtcatcttcgtctgccaattccttcaccgcagaaaagaagcaaagatcaccgtttttgtctattcttgtgtatcttctattgaaaaaacatgatgcaaagtaagcaatcaatcaactttttttttattca

SEQ ID NO: 52 - DNA, 23 bp, Artificial Sequence
  Primer
tgtcatcttcgtctgccaattcc

SEQ ID NO: 53 - DNA, 28 bp, Artificial Sequence
  Primer
acacaagaatagacaaaaacggtgatct

SEQ ID NO: 54 - DNA, 20 bp, Artificial Sequence
  Probe
tgcttcttttctgcggtgaa

SEQ ID NO: 55 - DNA, 21 bp, Artificial Sequence
  Probe
ttgcttcttttctacggtgaa

SEQ ID NO: 56 - DNA, 297 bp, Lactuca serriola
  misc_feature (66)..(66): n is a, c, g, or t
  misc_feature (101)..(101): n is a, c, g, or t
  misc_feature (143)..(143): n is a, c, g, or t
  misc_feature (153)..(155): n is a, c, g, or t
  misc_feature (174)..(174): n is a, c, g, or t
  misc_feature (243)..(243): n is a, c, g, or t
  misc_feature (247)..(247): n is a, c, g, or t
gctaaggcacagcctgatttagttgcagatgaaaacgatgatgaattactcacagaaaaagatagnttcgaggaggtgaaggatatggaacatgcaaagcngcaagaatctagcccaagtgatgctaaaaactctatcaaagnggaagaacannntgatgatgtttgtatgccnttaaaagatgatgaagatactatgaaggatgttgaagaggggactgatgttaagccctctgttgaaagntctnatttaagagatgttgcaaaagccattgataatcaagaaccagaagtggat

SEQ ID NO: 57 - DNA, 29 bp, Artificial Sequence
  Primer
cagatgaaaacgatgatgaattactcaca

SEQ ID NO: 58 - DNA, 24 bp, Artificial Sequence
  Primer
agcatcacttgggctagattcttg

SEQ ID NO: 59 - DNA, 17 bp, Artificial Sequence
  Probe
aggaggtgaaggatatg

SEQ ID NO: 60 - DNA, 17 bp, Artificial Sequence
  Probe
aggaggtgaatgatatg

SEQ ID NO: 61 - DNA, 949 bp, Lactuca serriola
  misc_feature (19)..(19): n is a, c, g, or t
  misc_feature (38)..(38): n is a, c, g, or t
  misc_feature (70)..(70): n is a, c, g, or t
  misc_feature (85)..(85): n is a, c, g, or t
  misc_feature (127)..(127): n is a, c, g, or t
  misc_feature (147)..(147): n is a, c, g, or t
  misc_feature (406)..(406): n is a, c, g, or t
  misc_feature (466)..(466): n is a, c, g, or t
  misc_feature (549)..(549): n is a, c, g, or t
  misc_feature (869)..(869): n is a, c, g, or t
  misc_feature (886)..(886): n is a, c, g, or t
cgcgggggaatggcttgantatgatgaaacggacggcnattcacgatattgaatacttttgtacccatcngaacctgccggaaanaatgcaccacttatcatcatcgtcgtggatgctccgccgctnttgctgtcatgcaacgcctnccttttcgccccctaccgccgttttatctacttctgctgctactctcactcctcccaagaagaaaaaactcgttttcatgggttctccctcggtaatctctcgcccaatgttcctacaatttacgttaagcatcgccatgggcaataattttcgattggggcttcgattttgaaatctgattcgtgttaggtctcggcttccgttctcgagactcttcttgacgcatcctccgccgctgattccttattcgaggttgcngcgattgttacccagccaccttcaggaagagataggggaagaaaagtgatgccatcaccngtagcacaacatgctctcgatagaggcttccctaatgacctaattttcacacctgttaaagccaatgaggaagcatttttgtncaatttcagagcacttgagcctcaactttgcatcacagcagcatatggcaacatattaccaaccaaatttttaaagattcctttattagggactgtgaatatacacccaagcttgttgcctttataccgtggagctgctcctgttcaaagagcattgcaggatggagttacagaaactggtgtatcattagcattcactatccgggcattagatgcgggccccattattgcctatgaaaaaaatgaaaatcgatgatcatattaaggctccagaattgcttgatctactatttgcacaaggatctaaactcttgcttcanaaacttcctctatattnaatggatctgcaaagacaaatgctcaagaacaagatgactcaaaagccactttggctccaaaa

SEQ ID NO: 62 - DNA, 24 bp, Artificial Sequence
  Primer
cgccatgggcaataattttcgatt

SEQ ID NO: 63 - DNA, 22 bp, Artificial Sequence
  Primer
gcgtcaagaagagtctcgagaa

SEQ ID NO: 64 - DNA, 16 bp, Artificial Sequence
  Probe
taggtctcggcttccg

SEQ ID NO: 65 - DNA, 17 bp, Artificial Sequence
  Probe
ttaggtctctgcttccg

SEQ ID NO: 66 - DNA, 201 bp, Lactuca serriola
ctttttactgttttatcaggaattaaktttttttagtaactatacccattccctgagtgtttgactacctattcttacctaacctatactacgtcgtgtgcaggattacatgcctagttttttgatggtccatagtttcattgataacaattataagttcaatattgattataaattatgcatcatgtttttggcattgtt

SEQ ID NO: 67 - DNA, 201 bp, Lactuca serriola
atattgggattggttcgttgaaatcgatttgaaaaatcagaaaaaattgatttgttctactagttgtaggaaacttgattttttgtaacctagtgtgacctttttttgcccctattgctttgtatagacactttttaggtagattttaacacaacactcaaaatgttctctaatataatatcatattatcggatattttca

SEQ ID NO: 68 - DNA, 201 bp, Lactuca serriola
atgattatgttggtttctaactcaaatccatcatcccatggtagatttgatgttggaatttctaaatctccacaaactctagattttctaatgataatgataatgtgataatctaactcttatatgattccattaccactaaggaatgtatgattgcaaatccttcttagaagagcacaattcaaacaatggtagaatcct

SEQ ID NO: 69 - DNA, 121 bp, Lactuca serriola
  misc_feature (85)..(85): n is a, c, g, or t
  misc_feature (103)..(103): n is a, c, g, or t
agcaagcatcgccgtcatcaatcctccggtacttgttccggcgatgacatcaaagtaatctgcaattcgtgcctcaggtccatcnatttcctgaagcttggantcgagaaatgaaagtatg

SEQ ID NO: 70 - DNA, 121 bp, Lactuca serriola
ttccagttctagttccagttccatcaatttcaaaggaattatggtgggaaatgcagtgacagattattactatgacaaccttggaactgtgacatattggtggagtcacgctatgatatct

SEQ ID NO: 71 - DNA, 27 bp, Artificial Sequence
  Primer
agttccagttccatcaatttcaaagga

SEQ ID NO: 72 - DNA, 25 bp, Artificial Sequence
  Primer
gtcacagttccaaggttgtcatagt

SEQ ID NO: 73 - DNA, 17 bp, Artificial Sequence
  Probe
tgcagtgacagattatt

SEQ ID NO: 74 - DNA, 15 bp, Artificial Sequence
  Probe
cagtgacggattatt

SEQ ID NO: 75 - DNA, 201 bp, Lactuca serriola
cattggcattagagatggtagtgaaataactatcatctcaaatcatcacactgtatgttgacatttactattttgtatgttgacatgtgtatagaatgatattttggtatgttctgttcataggatcttatggaagtagtttaataaagagtttcacatgctaagcatagacaatatgacaggtcaaccattaggtgtttc

SEQ ID NO: 76 - DNA, 121 bp, Lactuca serriola
  misc_feature (114)..(114): n is a, c, g, or t
cgacattacagccgcatcaaacgataacattcgcgattcttgaagcccgtgattcacttctggactattcgcaatctttgaagtcggtttaggagacgataaattcttgttttngtttcga

SEQ ID NO: 77 - DNA, 25 bp, Artificial Sequence
  Primer
gcatcaaacgataacattcgcgatt

SEQ ID NO: 78 - DNA, 25 bp, Artificial Sequence
  Primer
cgtctcctaaaccgacttcaaagat

SEQ ID NO: 79 - DNA, 20 bp, Artificial Sequence
  Probe
tgattcacttctggactatt

SEQ ID NO: 80 - DNA, 17 bp, Artificial Sequence
  Probe
ttcacttccggactatt

SEQ ID NO: 81 - DNA, 121 bp, Lactuca serriola
tttcacgtctgctgcatctgttgctaacctcgctgccactagactcgagttatgctcctcttcatcaaaccacccaacttcatttctcattatcgctgaaagcatcattcttcgaactcgt

SEQ ID NO: 82 - DNA, 19 bp, Artificial Sequence
  Primer
acctcgctgccactagact

SEQ ID NO: 83 - DNA, 27 bp, Artificial Sequence
  Primer
agaatgatgctttcagcgataatgaga

SEQ ID NO: 84 - DNA, 20 bp, Artificial Sequence
  Probe
agttatgctcctcttcatca

SEQ ID NO: 85 - DNA, 20 bp, Artificial Sequence
  Probe
agttatgctcctcctcatca

SEQ ID NO: 86 - DNA, 870 bp, Lactuca serriola
  misc_feature (148)..(148): n is a, c, g, or t
  misc_feature (157)..(157): n is a, c, g, or t
  misc_feature (270)..(270): n is a, c, g, or t
  misc_feature (327)..(327): n is a, c, g, or t
  misc_feature (394)..(394): n is a, c, g, or t
  misc_feature (425)..(425): n is a, c, g, or t
  misc_feature (572)..(572): n is a, c, g, or t
  misc_feature (601)..(601): n is a, c, g, or t
  misc_feature (658)..(658): n is a, c, g, or t
  misc_feature (723)..(723): n is a, c, g, or t
  misc_feature (725)..(725): n is a, c, g, or t
  misc_feature (747)..(747): n is a, c, g, or t
ggaaaaacggaaggacatagagttagagtgggagtttagaagcagaaggaagctatggcgtcagtgagagttgactcggaggtgactcggataatgatcggtgtgaacgagtcaagcatcaaaggatatccacatgcttcaattagtngcaaatcancatttgaatggactctgaacaagatcattcgctccaatacctccggttttaagctcctttttctccatgttcaagttcctgatgaagacggttttgatgatgttgatagtatntacgcctcaccacaagattttagagatgcaaatcgtaaagacaagattaatggatcncatttgctggagtactttgtgaacagatgtcatgatataggggttgtttgtgaagcatgggtgaagnggggtgatgccaaagaagtaatctgccatgnggtcaaaagagtcaaaccagacctccttgtagttggaaacagaggtcttggacccttccagagggtatttgtgggaactgtgagtgaattctgtgtgaagcactgtgaatgcccagttgtaacaatcaaacgcagtgcagaagaganccctaatgatcctgtagatgattgattgntcctctaaaagctactattaataatgtaaaatcttctctacaaccctctttcctggnttgtcttttttaatggagatttagctgtgtgtatctgtaagacctatgagttccttttttctagntnagttgttatacaactatgtttncaaggctgcttttgtgatatgtaactagattgacaagctttttagggatgaaatcacatttatgtcttttctactctctaacattacatcaaaaaatatattccttatatactcttgacaaaa

SEQ ID NO: 87 - DNA, 24 bp, Artificial Sequence
  Primer
tgtgagtgaattctgtgtgaagca

SEQ ID NO: 88 - DNA, 23 bp, Artificial Sequence
  Primer
cttctgcactgcgtttgattgtt

SEQ ID NO: 89 - DNA, 15 bp, Artificial Sequence
  Probe
caactgggcattcac

SEQ ID NO: 90 - DNA, 16 bp, Artificial Sequence
  Probe
acaactggacattcac

SEQ ID NO: 91 - DNA, 1917 bp, Lactuca serriola
  misc_feature (18)..(18): n is a, c, g, or t
  misc_feature (24)..(24): n is a, c, g, or t
  misc_feature (182)..(182): n is a, c, g, or t
  misc_feature (262)..(262): n is a, c, g, or t
  misc_feature (268)..(268): n is a, c, g, or t
  misc_feature (275)..(275): n is a, c, g, or t
  misc_feature (304)..(304): n is a, c, g, or t
  misc_feature (356)..(356): n is a, c, g, or t
  misc_feature (360)..(360): n is a, c, g, or t
  misc_feature (391)..(391): n is a, c, g, or t
  misc_feature (535)..(535): n is a, c, g, or t
  misc_feature (603)..(603): n is a, c, g, or t
  misc_feature (620)..(620): n is a, c, g, or t
  misc_feature (627)..(627): n is a, c, g, or t
  misc_feature (632)..(632): n is a, c, g, or t
  misc_feature (636)..(636): n is a, c, g, or t
  misc_feature (670)..(670): n is a, c, g, or t
  misc_feature (695)..(695): n is a, c, g, or t
  misc_feature (716)..(716): n is a, c, g, or t
  misc_feature (735)..(735): n is a, c, g, or t
  misc_feature (765)..(765): n is a, c, g, or t
  misc_feature (837)..(837): n is a, c, g, or t
  misc_feature (840)..(840): n is a, c, g, or t
  misc_feature (882)..(882): n is a, c, g, or t
  misc_feature (914)..(914): n is a, c, g, or t
  misc_feature (926)..(926): n is a, c, g, or t
  misc_feature (929)..(929): n is a, c, g, or t
  misc_feature (947)..(947): n is a, c, g, or t
  misc_feature (1101)..(1101): n is a, c, g, or t
  misc_feature (1104)..(1104): n is a, c, g, or t
  misc_feature (1109)..(1109): n is a, c, g, or t
  misc_feature (1111)..(1111): n is a, c, g, or t
  misc_feature (1116)..(1116): n is a, c, g, or t
  misc_feature (1124)..(1124): n is a, c, g, or t
  misc_feature (1153)..(1153): n is a, c, g, or t
  misc_feature (1215)..(1215): n is a, c, g, or t
  misc_feature (1221)..(1221): n is a, c, g, or t
  misc_feature (1227)..(1227): n is a, c, g, or t
  misc_feature (1241)..(1241): n is a, c, g, or t
  misc_feature (1246)..(1246): n is a, c, g, or t
  misc_feature (1251)..(1251): n is a, c, g, or t
  misc_feature (1284)..(1284): n is a, c, g, or t
  misc_feature (1291)..(1291): n is a, c, g, or t
  misc_feature (1297)..(1297): n is a, c, g, or t
  misc_feature (1305)..(1305): n is a, c, g, or t
  misc_feature (1318)..(1318): n is a, c, g, or t
  misc_feature (1321)..(1321): n is a, c, g, or t
  misc_feature (1346)..(1346): n is a, c, g, or t
  misc_feature (1348)..(1348): n is a, c, g, or t
  misc_feature (1350)..(1350): n is a, c, g, or t
  misc_feature (1366)..(1366): n is a, c, g, or t
  misc_feature (1395)..(1395): n is a, c, g, or t
  misc_feature (1400)..(1400): n is a, c, g, or t
  misc_feature (1405)..(1405): n is a, c, g, or t
  misc_feature (1407)..(1407): n is a, c, g, or t
  misc_feature (1413)..(1413): n is a, c, g, or t
  misc_feature (1419)..(1419): n is a, c, g, or t
  misc_feature (1432)..(1432): n is a, c, g, or t
  misc_feature (1444)..(1444): n is a, c, g, or t
  misc_feature (1447)..(1447): n is a, c, g, or t
  misc_feature (1477)..(1477): n is a, c, g, or t
  misc_feature (1497)..(1497): n is a, c, g, or t
  misc_feature (1502)..(1502): n is a, c, g, or t
  misc_feature (1512)..(1512): n is a, c, g, or t
  misc_feature (1515)..(1515): n is a, c, g, or t
  misc_feature (1521)..(1521): n is a, c, g, or t
  misc_feature (1527)..(1527): n is a, c, g, or t
  misc_feature (1530)..(1530): n is a, c, g, or t
  misc_feature (1545)..(1545): n is a, c, g, or t
  misc_feature (1558)..(1558): n is a, c, g, or t
  misc_feature (1584)..(1584): n is a, c, g, or t
  misc_feature (1591)..(1591): n is a, c, g, or t
  misc_feature (1593)..(1593): n is a, c, g, or t
  misc_feature (1601)..(1601): n is a, c, g, or t
  misc_feature (1612)..(1612): n is a, c, g, or t
  misc_feature (1614)..(1614): n is a, c, g, or t
  misc_feature (1621)..(1621): n is a, c, g, or t
  misc_feature (1625)..(1625): n is a, c, g, or t
  misc_feature (1627)..(1627): n is a, c, g, or t
  misc_feature (1636)..(1636): n is a, c, g, or t
  misc_feature (1644)..(1644): n is a, c, g, or t
  misc_feature (1661)..(1661): n is a, c, g, or t
  misc_feature (1666)..(1666): n is a, c, g, or t
  misc_feature (1682)..(1682): n is a, c, g, or t
  misc_feature (1689)..(1689): n is a, c, g, or t
  misc_feature (1698)..(1698): n is a, c, g, or t
  misc_feature (1701)..(1701): n is a, c, g, or t
  misc_feature (1706)..(1706): n is a, c, g, or t
  misc_feature (1716)..(1716): n is a, c, g, or t
  misc_feature (1729)..(1729): n is a, c, g, or t
  misc_feature (1735)..(1735): n is a, c, g, or t
  misc_feature (1742)..(1742): n is a, c, g, or t
  misc_feature (1747)..(1747): n is a, c, g, or t
  misc_feature (1753)..(1753): n is a, c, g, or t
  misc_feature (1755)..(1755): n is a, c, g, or t
  misc_feature (1758)..(1758): n is a, c, g, or t
  misc_feature (1765)..(1765): n is a, c, g, or t
  misc_feature (1768)..(1768): n is a, c, g, or t
  misc_feature (1775)..(1775): n is a, c, g, or t
  misc_feature (1777)..(1777): n is a, c, g, or t
  misc_feature (1784)..(1784): n is a, c, g, or t
  misc_feature (1786)..(1786): n is a, c, g, or t
  misc_feature (1791)..(1791): n is a, c, g, or t
  misc_feature (1807)..(1807): n is a, c, g, or t
  misc_feature (1818)..(1818): n is a, c, g, or t
  misc_feature (1821)..(1821): n is a, c, g, or t
  misc_feature (1828)..(1828): n is a, c, g, or t
  misc_feature (1830)..(1830): n is a, c, g, or t
  misc_feature (1837)..(1837): n is a, c, g, or t
  misc_feature (1847)..(1847): n is a, c, g, or t
  misc_feature (1850)..(1850): n is a, c, g, or t
  misc_feature (1914)..(1914): n is a, c, g, or t
gcggggggcgacgatttngggggncaagttgatttccttatactttacttcaaaatcttctccatagttgaattgctgataatcagttcagaagcttgtttgctgcatttcctggtgtatggcaccaatgaagggcattctttctctgcaaagggctgttctatcaaggcatcaaaatgcanactgggggataaatgctaccggctagacttttcagcacgcagtctgcgacaaccgccaccaccgcccaaccaccaccgcnaccacntccaccngaaaaaacccactttggtggcctgaaagntgaagaccgcatcttcacaaacctatacggtttacacgacccctttctcaanggcncaatgaaacgtggcgattggcatagaactanagacatagtaatcaaaggtgctgattggatagtaaacgaaatgaaaaaatccggcttacgtggacgtggaggtgctggtttcccatcagggctaaaatggtcattcatgccaaaagtatccgatggtcgtccatcttatcttgntgtaaacgcagacgaaagtgaacccggaacttgcaaagatagagaaatcatgcgtaacgatccacacnagcttctagaaggatgnttaatanctggngtangtatgcgtgcaaccgctgcctacatttacatcangggcgaatacgtaaatgaacgtttnaatttagaaaaagcaagaaangaagcatatgcagctggantacttggaaaaaacgcgtgtgggtccgggnatgatttcgatgtccatatccatttcggagccggagcctacatttgtggtgaagaaaccgcgcttctcgaanccntcgagggcaaacaaggaaaaccgcgtttgaagccgccttttnccgccaacgcggggttatacgggtgtcccacnaccgtcacaaangtngaaacaatcgcggtgtcnccgactattctaagacgtgggcccgagtggttttctagctttggtagaaagaacattcggggactaaacttttctgtatatcgggtcatgtgaacaaaccgtgtacagtggaagaggagatgagtattccattgaaggagttgttggagcggcnttntggcngnttgangggcggangggacaatttgctagcggtgattccgggnggttcttctgttcctttgcttacaaaggatttatgcgaagacgtgttgatggattttgatgngttganagctgntcaatctggattanggacngctgntgttattgtgatggataagtcgactgatattgnggatgcnattgcnaggctttngtatttttataancangagagttgtggtcagtgtacgcctngnanggagggaactgggtgnctttggatgattatggaaaggatgaaagntgggnatgcnanattggnggagantgatatgcttcangaagtgactaancanattgaagggcatactatttgtgcacttggngatgctgctgcttggcctgntcaanggcttattanacnttttangcctgnganggagaggaggatcanggagcgtgctgancgggagttgcttcaagcagctgcttnaaatcangntgaatggnttcctacctgnangaaaacntgangngactttggnctttggancataatatgattaatgnttaangtttgtgttgctgttnaactacnatgtgattnaanacagnacccttctcnttagattgggggnaacttntgtgtgnttaangatacnanganatcctantgntattatngnacttcantnagccntatgcttttggacacntgtcaaaatgntantaagccnantgcattnttgtaatcanacnatggaagcttttcataagctcaagtttcatgccttgtcagaacattaaccgttggtggtttggngaa

SEQ ID NO: 92 - DNA, 26 bp, Artificial Sequence
  Primer
aaaggtgctgattggatagtaaacga

SEQ ID NO: 93 - DNA, 23 bp, Artificial Sequence
  Primer
attttagccctgatgggaaacca

SEQ ID NO: 94 - DNA, 16 bp, Artificial Sequence
  Probe
cacgtaagccggattt

SEQ ID NO: 95 - DNA, 16 bp, Artificial Sequence
  Probe
cacgtaagccagattt